European Patent Specification EP 3 802 599 B1, published December 20, 2023. Title: BISPECIFIC ANTIBODIES AGAINST CEACAM5 AND CD47. Applicant: LamKap Bio beta Ltd. The sequence listing filed with the application follows.

SEQUENCE LISTING (116 sequences)

SEQ ID NO: 1 - protein, 8 aa, Artificial Sequence
  Mab CD47 CDRH1
GFTFSSYA

SEQ ID NO: 2 - protein, 8 aa, Artificial Sequence
  Mab CD47 CDRH2
ISGSGGST

SEQ ID NO: 3 - protein, 9 aa, Artificial Sequence
  Mab CD47 CDRH3
AKSYGAFDY

SEQ ID NO: 4 - protein, 116 aa, Artificial Sequence
  Mab CD47 VH
EVQLLESGGGLVQPGGSLRLSCAASGFTFSSYAMSWVRQAPGKGLEWVSAISGSGGSTYYADSVKGRFTISRDNSKNTLYLQMNSLRAEDTAVYYCAKSYGAFDYWGQGTLVTVSS

SEQ ID NO: 5 - protein, 445 aa, Artificial Sequence
  Mab CD47 HC
EVQLLESGGGLVQPGGSLRLSCAASGFTFSSYAMSWVRQAPGKGLEWVSAISGSGGSTYYADSVKGRFTISRDNSKNTLYLQMNSLRAEDTAVYYCAKSYGAFDYWGQGTLVTVSSASTKGPSVFPLAPSSKSTSGGTAALGCLVKDYFPEPVTVSWNSGALTSGVHTFPAVLQSSGLYSLSSVVTVPSSSLGTQTYICNVNHKPSNTKVDKRVEPKSCDKTHTCPPCPAPELLGGPSVFLFPPKPKDTLMISRTPEVTCVVVDVSHEDPEVKFNWYVDGVEVHNAKTKPREEQYNSTYRVVSVLTVLHQDWLNGKEYKCKVSNKALPAPIEKTISKAKGQPREPQVYTLPPSREEMTKNQVSLTCLVKGFYPSDIAVEWESNGQPENNYKTTPPVLDSDGSFFLYSKLTVDKSRWQQGNVFSCSVMHEALHNHYTQKSLSLSPG

SEQ ID NO: 6 - DNA, 1338 bp, Artificial Sequence
  Mab CD47 HC
gaggtgcagctgttggagtctgggggaggcttggtacagcctggggggtccctgagactctcctgtgcagcctctggattcacctttagcagctatgccatgagctgggtccgccaggctccagggaaggggctggagtgggtctcagctattagtggtagtggtggtagcacatactacgcagactccgtgaagggccggttcaccatctccagagacaattccaagaacacgctgtatctgcaaatgaacagcctgagagccgaggacacggccgtatattactgtgcgaaaagttatggtgcttttgactactggggccagggaaccctggtcacagtctcgagcgcctccaccaagggcccatcggtcttccccctggcaccctcctccaagagcacctctgggggcacagcggccctgggctgcctggtcaaggactacttccccgaaccggtgacagtctcgtggaactcaggagccctgaccagcggcgtgcacaccttcccggctgtcctacagtcctcaggactctactccctcagcagcgtggtgactgtgccctccagcagcttgggcacccagacctacatctgcaacgtgaatcacaagcccagcaacaccaaggtggacaagagagttgagcccaaatcttgtgacaaaactcacacatgcccaccgtgcccagcacctgaactcctggggggaccgtcagtcttcctcttccccccaaaacccaaggacaccctcatgatctcccggacccctgaggtcacatgcgtggtggtggacgtgagccacgaagaccctgaggtcaagttcaactggtacgtggacggcgtggaggtgcataatgccaagacaaagccgcgggaggagcagtacaacagcacgtaccgtgtggtcagcgtcctcaccgtcctgcaccaggactggctgaatggcaaggagtacaagtgcaaggtctccaacaaagccctcccagcccccatcgagaaaaccatctccaaagccaaagggcagccccgagaaccacaggtgtataccctgcccccatctcgggaggagatgaccaagaaccaggtcagcctgacttgcctggtcaaaggcttctatcccagcgacatcgccgtggagtgggagagcaacgggcagccggagaacaactacaagaccacgcctcccgtgctggactccgacggctccttcttcctctatagcaagctcaccgtggacaagtccaggtggcagcaggggaacgtcttctcatgctccgtgatgcatgaggctctgcacaaccactacacgcagaagagcctctccctgtctccgggttaa

SEQ ID NO: 7 - protein, 6 aa, Artificial Sequence
  Mab CD47 CDRL1
QSISSY

SEQ ID NO: 8 - protein, 4 aa, Artificial Sequence
  MabCd47 CDRL2
AASS

SEQ ID NO: 9 - protein, 10 aa, Artificial Sequence
  Mab CD47 CDRL3
QQMHPRAPKT

SEQ ID NO: 10 - protein, 108 aa, Artificial Sequence
  Mab CD47 VL
DIQMTQSPSSLSASVGDRVTITCRASQSISSYLNWYQQKPGKAPKLLIYAASSLQSGVPSRFSGSGSGTDFTLTISSLQPEDFATYYCQQMHPRAPKTFGQGTKVEIK

SEQ ID NO: 11 - protein, 215 aa, Artificial Sequence
  Mab CD47 LC
DIQMTQSPSSLSASVGDRVTITCRASQSISSYLNWYQQKPGKAPKLLIYAASSLQSGVPSRFSGSGSGTDFTLTISSLQPEDFATYYCQQMHPRAPKTFGQGTKVEIKRTVAAPSVFIFPPSDEQLKSGTASVVCLLNNFYPREAKVQWKVDNALQSGNSQESVTEQDSKDSTYSLSSTLTLSKADYEKHKVYACEVTHQGLSSPVTKSFNRGEC

SEQ ID NO: 12 - DNA, 648 bp, Artificial Sequence
  Mab CD47 LC
gacatccagatgacccagtctccatcctccctgtctgcatctgtaggagacagagtcaccatcacttgccgggcaagtcagagcattagcagctatttaaattggtatcagcagaaaccagggaaagcccctaagctcctgatctatgctgcatccagtttgcaaagtggggtcccatcaaggttcagtggcagtggatctgggacagatttcactctcaccatcagcagtctgcaacctgaagattttgcaacttactactgtcagcagatgcacccgcgcgccccgaagaccttcggccaagggaccaaggtggaaatcaaacgtacggtggctgcaccatctgtcttcatcttcccgccatctgatgagcagttgaaatctggaactgcctctgttgtgtgcctgctgaataacttctatcccagagaggccaaagtacagtggaaggtggataacgccctccaatcgggtaactcccaggagagtgtcacagagcaggacagcaaggacagcacctacagcctcagcagcaccctgacgctgagcaaagcagactacgagaaacacaaagtctacgcctgcgaagtcacccatcagggcctgagctcgcccgtcacaaagagcttcaacaggggagagtgttaa

SEQ ID NO: 13 - protein, 116 aa, Artificial Sequence
  Mab CEA CL
FGGGTKLTVLGQPKAAPSVTLFPPSSEELQANKATLVCLISDFYPGAVTVAWKADSSPVKAGVETTTPSKQSNNKYAASSYLSLTPEQWKSHRSYSCQVTHEGSTVEKTVAPTECS

SEQ ID NO: 14 - DNA, 24 bp, Artificial Sequence
  Primer
gtctgaagcattatgtgttgaagc

SEQ ID NO: 15 - DNA, 23 bp, Artificial Sequence
  Primer
gtgagtacattcattgtactgtg

SEQ ID NO: 16 - DNA, 24 bp, Artificial Sequence
  Primer
ttgtgtgactcttaactctcagag

SEQ ID NO: 17 - DNA, 25 bp, Artificial Sequence
  Primer
gaggccacttgtgtagcgccaagtg

SEQ ID NO: 18 - DNA, 21 bp, Artificial Sequence
  Primer
gtgagtccatggctgtcactg

SEQ ID NO: 19 - DNA, 20 bp, Artificial Sequence
  Primer
cctgacttggctattctcag

SEQ ID NO: 20 - protein, 121 aa, Artificial Sequence
  Mab CEA variable heavy chain
QVQLVQSGAEVKKPGASVKVSCKASGYTFTEFGMNWVRQAPGQGLEWMGWINTKTGEATYVEEFKGRVTFTTDTSTSTAYMELRSLRSDDTAVYYCARWDFAYYVEAMDYWGQGTTVTVSS

SEQ ID NO: 21 - protein, 108 aa, Artificial Sequence
  Mab CEA variable light chain
DIQMTQSPSSLSASVGDRVTITCKASAAVGTYVAWYQQKPGKAPKLLIYSASYRKRGVPSRFSGSGSGTDFTLTISSLQPEDFATYYCHQYYTYPLFTFGQGTKLEIK

SEQ ID NO: 22 - protein, 5 aa, Artificial Sequence
  Epitope of CD3 epsilon
QDGNE

SEQ ID NO: 23 - protein, 445 aa, Artificial Sequence
  Mab CD47 HC-DE
EVQLLESGGGLVQPGGSLRLSCAASGFTFSSYAMSWVRQAPGKGLEWVSAISGSGGSTYYADSVKGRFTISRDNSKNTLYLQMNSLRAEDTAVYYCAKSYGAFDYWGQGTLVTVSSASTKGPSVFPLAPSSKSTSGGTAALGCLVKDYFPEPVTVSWNSGALTSGVHTFPAVLQSSGLYSLSSVVTVPSSSLGTQTYICNVNHKPSNTKVDKRVEPKSCDKTHTCPPCPAPELLGGPDVFLFPPKPKDTLMISRTPEVTCVVVDVSHEDPEVKFNWYVDGVEVHNAKTKPREEQYNSTYRVVSVLTVLHQDWLNGKEYKCKVSNKALPAPEEKTISKAKGQPREPQVYTLPPSREEMTKNQVSLTCLVKGFYPSDIAVEWESNGQPENNYKTTPPVLDSDGSFFLYSKLTVDKSRWQQGNVFSCSVMHEALHNHYTQKSLSLSPG

SEQ ID NO: 24 - protein, 445 aa, Artificial Sequence
  Mab CD47 HC-DEA
EVQLLESGGGLVQPGGSLRLSCAASGFTFSSYAMSWVRQAPGKGLEWVSAISGSGGSTYYADSVKGRFTISRDNSKNTLYLQMNSLRAEDTAVYYCAKSYGAFDYWGQGTLVTVSSASTKGPSVFPLAPSSKSTSGGTAALGCLVKDYFPEPVTVSWNSGALTSGVHTFPAVLQSSGLYSLSSVVTVPSSSLGTQTYICNVNHKPSNTKVDKRVEPKSCDKTHTCPPCPAPELLAGPDVFLFPPKPKDTLMISRTPEVTCVVVDVSHEDPEVKFNWYVDGVEVHNAKTKPREEQYNSTYRVVSVLTVLHQDWLNGKEYKCKVSNKALPAPEEKTISKAKGQPREPQVYTLPPSREEMTKNQVSLTCLVKGFYPSDIAVEWESNGQPENNYKTTPPVLDSDGSFFLYSKLTVDKSRWQQGNVFSCSVMHEALHNHYTQKSLSLSPG

SEQ ID NO: 25 - protein, 5 aa, Artificial Sequence
  Mab CD47 CDRH1
SYAMS

SEQ ID NO: 26 - protein, 17 aa, Artificial Sequence
  Mab CD47 CHRH2
AISGSGGSTYYADSVKG

SEQ ID NO: 27 - protein, 7 aa, Artificial Sequence
  Mab CD47 CDRH3
SYGAFDY

SEQ ID NO: 28 - protein, 11 aa, Artificial Sequence
  Mab CD47 CDRL1; KA3
RASQSISSYLN

SEQ ID NO: 29 - protein, 7 aa, Artificial Sequence
  Mab CD47 CDRL2; KA3
AASSLQS

SEQ ID NO: 30 - protein, 10 aa, Artificial Sequence
  Mab CD47 CDRL3; KA3
QQMHPRAPKT

SEQ ID NO: 31 - protein, 13 aa, Artificial Sequence
  Mab CEA CDRL1; 1D9 (AC5)
SGSSSNIGYGLVS

SEQ ID NO: 32 - protein, 7 aa, Artificial Sequence
  Mab CEA CDRL2; 1D9 (AC5)
AGNLRPS

SEQ ID NO: 33 - protein, 10 aa, Artificial Sequence
  Mab CEA CDRL3; 1D9 (AC5)
GTWDFNYGVV

SEQ ID NO: 34 - protein, 13 aa, Artificial Sequence
  Mab CEA CDRL1; 1G6 (AC22)
SGSSSNIANGIVS

SEQ ID NO: 35 - protein, 7 aa, Artificial Sequence
  Mab CEA CDRL2; 1G6 (AC22)
FDNLRPS

SEQ ID NO: 36 - protein, 10 aa, Artificial Sequence
  Mab CEA CDRL3; 1G6 (AC22)
GTWDFSYGIV

SEQ ID NO: 37 - protein, 14 aa, Artificial Sequence
  Mab CEA CDRL1; 1D5 (AC10)
TGSSSNIYANSNVH

SEQ ID NO: 38 - protein, 7 aa, Artificial Sequence
  Mab CEA CDRL2; 1D5 (AC10)
SGSNRPS

SEQ ID NO: 39 - protein, 13 aa, Artificial Sequence
  Mab CEA CDRL3; 1D5 (AC10)
QSYDPAHNLLTAV

SEQ ID NO: 40 - protein, 14 aa, Artificial Sequence
  Mab CEA CDRL1, 2B8 (AC13)
TGTSSNVRYAAGVS

SEQ ID NO: 41 - protein, 7 aa, Artificial Sequence
  Mab CEA CDRL2; 2B8 (AC13)
EVSNRPS

SEQ ID NO: 42 - protein, 13 aa, Artificial Sequence
  Mab CEA CDRL3; 2B8 (AC13)
SSWDFEHGPAAKV

SEQ ID NO: 43 - protein, 11 aa, Artificial Sequence
  Mab CEA CDRL1; 1A2 (AC18)
GGNGIGDASVH

SEQ ID NO: 44 - protein, 7 aa, Artificial Sequence
  Mab CEA CDRL2; 1A2 (AC18)
STTTRPS

SEQ ID NO: 45 - protein, 13 aa, Artificial Sequence
  Mab CEA CDRL3; 1A2 (AC18)
QVWDGFGPRHRAV

SEQ ID NO: 46 - protein, 13 aa, Artificial Sequence
  Mab CEA CDRL1; 1A8 (AC23)
SGSSSNIGYGLVN

SEQ ID NO: 47 - protein, 7 aa, Artificial Sequence
  Mab CEA CDRL2; 1A8 (AC23)
ATNTRPS

SEQ ID NO: 48 - protein, 10 aa, Artificial Sequence
  Mab CEA CDRL3; 1A8 (AC23)
AAWDFSYKVV

SEQ ID NO: 49 - protein, 13 aa, Artificial Sequence
  Mab CEA CDRL1; 2F4 (AC25)
SGSSSNIGITPVS

SEQ ID NO: 50 - protein, 7 aa, Artificial Sequence
  Mab CEA CDRL2; 2F4 (AC25)
SNNFRPS

SEQ ID NO: 51 - protein, 13 aa, Artificial Sequence
  Mab CEA CDRL3; 2F4 (AC25)
GTWDRTGHEIRPV

SEQ ID NO: 52 - protein, 14 aa, Artificial Sequence
  Mab CEA CDRL1; 2F7 (AC26)
TGTSSDVKYANAVS

SEQ ID NO: 53 - protein, 7 aa, Artificial Sequence
  Mab CEA CDRL2; 2F7 (AC26)
SNSIRPS

SEQ ID NO: 54 - protein, 13 aa, Artificial Sequence
  Mab CEA CDRL3; 2F7 (AC26)
SSYDPRGNLLIRV

SEQ ID NO: 55 - protein, 14 aa, Artificial Sequence
  Mab CEA CDRL1; 2C11 (AC27)
TGSSSNIGYADKVH

SEQ ID NO: 56 - protein, 7 aa, Artificial Sequence
  Mab CEA CDRL2; 2C11 (AC27)
NNSDRPS

SEQ ID NO: 57 - protein, 12 aa, Artificial Sequence
  Mab CEA CDRL3; 2C11 (AC27)
QSYDGYNMLTAV

SEQ ID NO: 58 - protein, 13 aa, Artificial Sequence
  Mab CEA CDRL1; C11 (AC28)
TRSSGSINDITVH

SEQ ID NO: 59 - protein, 7 aa, Artificial Sequence
  Mab CEA CDRL2; C11 (AC28)
GYNARPS

SEQ ID NO: 60 - protein, 11 aa, Artificial Sequence
  Mab CEA CDRL3; C11 (AC28)
QSWDGHGSAYV

SEQ ID NO: 61 - protein, 14 aa, Artificial Sequence
  Mab CEA CDRL1; 2B5 (AC29)
TGTSSDVEFTNGVS

SEQ ID NO: 62 - protein, 7 aa, Artificial Sequence
  Mab CEA CDRL2; 2B5 (AC29)
GFSSRPS

SEQ ID NO: 63 - protein, 13 aa, Artificial Sequence
  Mab CEA CDRL3; 2B5 (AC29)
SSYDPPWHLLARV

SEQ ID NO: 64 - protein, 215 aa, Artificial Sequence
  Mab CEA 1D9 VLCL2 CEA (AC5)
QSVLTQPPSVSAAPGQKVTISCSGSSSNIGYGLVSWYQQLPGTAPKLLIYAGNLRPSGIPDRFSGSKSGTSATLGITGLQTGDEADYYCGTWDFNYGVVFGGGTKLTVLGQPKAAPSVTLFPPSSEELQANKATLVCLISDFYPGAVTVAWKADSSPVKAGVETTTPSKQSNNKYAASSYLSLTPEQWKSHRSYSCQVTHEGSTVEKTVAPTECS

SEQ ID NO: 65 - protein, 215 aa, Artificial Sequence
  Mab CEA 1G6 VLCL2 CEA (AC22)
QSVLTQPPSVSAAPGQKVTISCSGSSSNIANGIVSWYQQLPGTAPKLLIYFDNLRPSGIPDRFSGSKSGTSATLGITGLQTGDEADYYCGTWDFSYGIVFGGGTKLTVLGQPKAAPSVTLFPPSSEELQANKATLVCLISDFYPGAVTVAWKADSSPVKAGVETTTPSKQSNNKYAASSYLSLTPEQWKSHRSYSCQVTHEGSTVEKTVAPTECS

SEQ ID NO: 66 - protein, 219 aa, Artificial Sequence
  Mab CEA 1D5 VLCL2 CEA (AC10)
QSVLTQPPSVSGAPGQRVTISCTGSSSNIYANSNVHWYQQLPGTAPKLLIYSGSNRPSGVPDRFSGSKSGTSASLAITGLQAEDEADYYCQSYDPAHNLLTAVFGGGTKLTVLGQPKAAPSVTLFPPSSEELQANKATLVCLISDFYPGAVTVAWKADSSPVKAGVETTTPSKQSNNKYAASSYLSLTPEQWKSHRSYSCQVTHEGSTVEKTVAPTECS

SEQ ID NO: 67 - protein, 219 aa, Artificial Sequence
  Mab CEA 2B8 VLCL2 CEA (AC13)
QSALTQPASVSGSPGQSITISCTGTSSNVRYAAGVSWYQQHPGKAPKLMIYEVSNRPSGVSNRFSGSKSGNTASLTISGLQAEDEADYYCSSWDFEHGPAAKVFGGGTKLTVLGQPKAAPSVTLFPPSSEELQANKATLVCLISDFYPGAVTVAWKADSSPVKAGVETTTPSKQSNNKYAASSYLSLTPEQWKSHRSYSCQVTHEGSTVEKTVAPTECS

SEQ ID NO: 68 - protein, 216 aa, Artificial Sequence
  Mab CEA 1A2 VLCL2 CEA (AC18)
SYVLTQPPSVSVAPGKTARITCGGNGIGDASVHWYQQKPGQAPVLVIYSTTTRPSGIPERFSGSNSGNTATLTISRVEAGDEADYYCQVWDGFGPRHRAVFGGGTKLTVLGQPKAAPSVTLFPPSSEELQANKATLVCLISDFYPGAVTVAWKADSSPVKAGVETTTPSKQSNNKYAASSYLSLTPEQWKSHRSYSCQVTHEGSTVEKTVAPTECS

SEQ ID NO: 69 - protein, 215 aa, Artificial Sequence
  Mab CEA 1A8 VLCL2 CEA (AC23)
QSVLTQPPSASGTPGQRVTISCSGSSSNIGYGLVNWYQQLPGTAPKLLIYATNTRPSGVPDRFSGSKSGTSASLAISGLQSEDEADYYCAAWDFSYKVVFGGGTKLTVLGQPKAAPSVTLFPPSSEELQANKATLVCLISDFYPGAVTVAWKADSSPVKAGVETTTPSKQSNNKYAASSYLSLTPEQWKSHRSYSCQVTHEGSTVEKTVAPTECS

SEQ ID NO: 70 - protein, 218 aa, Artificial Sequence
  Mab CEA 2F4 VLCL2 CEA (AC25)
QSVLTQPPSVSAAPGQKVTISCSGSSSNIGITPVSWYQQLPGTAPKLLIYSNNFRPSGIPDRFSGSKSGTSATLGITGLQTGDEADYYCGTWDRTGHEIRPVFGGGTKLTVLGQPKAAPSVTLFPPSSEELQANKATLVCLISDFYPGAVTVAWKADSSPVKAGVETTTPSKQSNNKYAASSYLSLTPEQWKSHRSYSCQVTHEGSTVEKTVAPTECS

SEQ ID NO: 71 - protein, 219 aa, Artificial Sequence
  Mab CEA 2F4 VLCL2 CEA (AC25)
QSALTQPASVSGSPGQSITISCTGTSSDVKYANAVSWYQQHPGKAPKLMIYSNSIRPSGVSNRFSGSKSGNTASLTISGLQAEDEADYYCSSYDPRGNLLIRVFGGGTKLTVLGQPKAAPSVTLFPPSSEELQANKATLVCLISDFYPGAVTVAWKADSSPVKAGVETTTPSKQSNNKYAASSYLSLTPEQWKSHRSYSCQVTHEGSTVEKTVAPTECS

SEQ ID NO: 72 - protein, 218 aa, Artificial Sequence
  Mab CEA 2C11 VLCL2 CEA
QSVLTQPPSVSGAPGQRVTISCTGSSSNIGYADKVHWYQQLPGTAPKLLIYNNSDRPSGVPDRFSGSKSGTSASLAITGLQAEDEADYYCQSYDGYNMLTAVFGGGTKLTVLGQPKAAPSVTLFPPSSEELQANKATLVCLISDFYPGAVTVAWKADSSPVKAGVETTTPSKQSNNKYAASSYLSLTPEQWKSHRSYSCQVTHEGSTVEKTVAPTECS

SEQ ID NO: 73 - protein, 218 aa, Artificial Sequence
  Mab CEA C11 VLCL2 CEA (AC28)
NFMLTQPHSVSESPGKTVTISCTRSSGSINDITVHWYQQRPGSSPTTVIYGYNARPSGVPDRFSGSIDSSSNSASLTISGLKTEDEADYYCQSWDGHGSAYVFGGGTKLTVLGQPKAAPSVTLFPPSSEELQANKATLVCLISDFYPGAVTVAWKADSSPVKAGVETTTPSKQSNNKYAASSYLSLTPEQWKSHRSYSCQVTHEGSTVEKTVAPTECS

SEQ ID NO: 74 - protein, 219 aa, Artificial Sequence
  Mab CEA 2B5 VLCL2 CEA (AC29)
QSALTQPASVSGSPGQSITISCTGTSSDVEFTNGVSWYQQHPGKAPKLMIYGFSSRPSGVSNRFSGSKSGNTASLTISGLQAEDEADYYCSSYDPPWHLLARVFGGGTKLTVLGQPKAAPSVTLFPPSSEELQANKATLVCLISDFYPGAVTVAWKADSSPVKAGVETTTPSKQSNNKYAASSYLSLTPEQWKSHRSYSCQVTHEGSTVEKTVAPTECS

SEQ ID NO: 75 - DNA, 648 bp, Artificial Sequence
  Nucleic acid 1D9 VLCL2 CEA (AC5)
cagtctgtgttgacgcagccgccctcagtgtctgcggccccaggacagaaggtcaccatctcctgctctggaagcagctccaacattggttatgggcttgtatcctggtaccagcagctcccaggaacagcccccaaactcctcatttatgctggtaatcttcgaccctcagggattcctgaccgattctctggctccaagtctggcacgtcagccaccctgggcatcaccggactccagactggggacgaggccgattattactgcggaacatgggattttaattatggggttgtgttcggcggagggaccaagctgaccgtcctaggtcagcccaaggctgccccctcggtcactctgttcccgccctcctctgaggagcttcaagccaacaaggccacactggtgtgtctcataagtgacttctacccgggagccgtgacagtggcttggaaagcagatagcagccccgtcaaggcgggagtggagaccaccacaccctccaaacaaagcaacaacaagtacgcggccagcagctatctgagcctgacgcctgagcagtggaagtcccacagaagctacagctgccaggtcacgcatgaagggagcaccgtggagaagacagtggcccctacagaatgttcataa

SEQ ID NO: 76 - DNA, 648 bp, Artificial Sequence
  Nucleic acid 1G6 VLCL2 CEA (AC22)
cagtctgtgttgacgcagccgccctcagtgtctgcggccccaggacagaaggtcaccatctcctgctctggaagcagctccaacattgctaatgggattgtatcctggtaccagcagctcccaggaacagcccccaaactcctcatttattttgataatcttcgaccctcagggattcctgaccgattctctggctccaagtctggcacgtcagccaccctgggcatcaccggactccagactggggacgaggccgattattactgcggaacatgggattttagttatggtattgtgttcggcggagggaccaagctgaccgtcctaggtcagcccaaggctgccccctcggtcactctgttcccgccctcctctgaggagcttcaagccaacaaggccacactggtgtgtctcataagtgacttctacccgggagccgtgacagtggcttggaaagcagatagcagccccgtcaaggcgggagtggagaccaccacaccctccaaacaaagcaacaacaagtacgcggccagcagctatctgagcctgacgcctgagcagtggaagtcccacagaagctacagctgccaggtcacgcatgaagggagcaccgtggagaagacagtggcccctacagaatgttcataa

SEQ ID NO: 77 - DNA, 660 bp, Artificial Sequence
  Nucleic acid 1D5 VLCL2 CEA (AC10)
cagtctgtgctgacgcagccgccctcagtgtctggggccccagggcagagggtcaccatctcctgcactgggagcagctccaacatctatgcgaatagtaatgtacactggtaccagcagcttccaggaacagcccccaaactcctcatctattctggtagcaatcggccctcaggggtccctgaccgattctctggctccaagtctggcacctcagcctccctggccatcactgggctccaggctgaggatgaggctgattattactgccagtcctatgatcccgcgcacaacttgctcactgctgtgttcggcggagggaccaagctgaccgtcctaggtcagcccaaggctgccccctcggtcactctgttcccgccctcctctgaggagcttcaagccaacaaggccacactggtgtgtctcataagtgacttctacccgggagccgtgacagtggcttggaaagcagatagcagccccgtcaaggcgggagtggagaccaccacaccctccaaacaaagcaacaacaagtacgcggccagcagctatctgagcctgacgcctgagcagtggaagtcccacagaagctacagctgccaggtcacgcatgaagggagcaccgtggagaagacagtggcccctacagaatgttcataa

SEQ ID NO: 78 - DNA, 660 bp, Artificial Sequence
  Nucleic acid 2B8 VLCL2 CEA (AC13)
cagtctgccctgactcagcctgcctccgtgtctgggtctcctggacagtcgatcaccatctcctgcactggaaccagcagtaatgttaggtatgctgctggtgtctcctggtaccaacagcacccaggcaaagcccccaaactcatgatttatgaggtcagtaatcggccctcaggggtttctaatcgcttctctggctccaagtctggcaacacggcctccctgaccatctctgggctccaggctgaggacgaggctgattattactgcagctcatgggattttgagcatggtcctgctgctaaggtgttcggcggagggaccaagctgaccgtcctaggtcagcccaaggctgccccctcggtcactctgttcccgccctcctctgaggagcttcaagccaacaaggccacactggtgtgtctcataagtgacttctacccgggagccgtgacagtggcttggaaagcagatagcagccccgtcaaggcgggagtggagaccaccacaccctccaaacaaagcaacaacaagtacgcggccagcagctatctgagcctgacgcctgagcagtggaagtcccacagaagctacagctgccaggtcacgcatgaagggagcaccgtggagaagacagtggcccctacagaatgttcataa

SEQ ID NO: 79 - DNA, 651 bp, Artificial Sequence
  Nucleic acid 1A2 VLCL2 CEA
tcctatgtgctgactcagccaccctcagtgtcagtggccccaggaaagacggccaggattacctgtgggggaaacggtattggagatgcgtctgtgcactggtaccagcagaagccaggccaggcccctgtgctggtcatctattctactactacgcggccctcagggattcctgagcgattctctggctccaactctgggaacacggccaccctgaccatcagcagggtcgaagccggggatgaggccgactattactgtcaggtgtgggatgggtttggtcctaggcatagggctgtgttcggcggagggaccaagctgaccgtcctaggtcagcccaaggctgccccctcggtcactctgttcccgccctcctctgaggagcttcaagccaacaaggccacactggtgtgtctcataagtgacttctacccgggagccgtgacagtggcttggaaagcagatagcagccccgtcaaggcgggagtggagaccaccacaccctccaaacaaagcaacaacaagtacgcggccagcagctatctgagcctgacgcctgagcagtggaagtcccacagaagctacagctgccaggtcacgcatgaagggagcaccgtggagaagacagtggcccctacagaatgttcataa

SEQ ID NO: 80 - DNA, 648 bp, Artificial Sequence
  Nucleic acid 1A8 VLCL2 CEA (AC23)
cagtctgtgctgactcagccaccctcagcgtctgggacccccgggcagagggtcaccatctcttgttctggaagcagctccaacatcgggtatgggcttgtaaactggtaccagcagctcccaggaacggcccccaaactcctcatctatgctactaatacgcggccctcaggggtccctgaccgattctctggctccaagtctggcacctcagcctccctggccatcagtgggctccagtctgaggatgaggctgattattactgtgcagcatgggattttagttataaggttgtgttcggcggagggaccaagctgaccgtcctaggtcagcccaaggctgccccctcggtcactctgttcccgccctcctctgaggagcttcaagccaacaaggccacactggtgtgtctcataagtgacttctacccgggagccgtgacagtggcttggaaagcagatagcagccccgtcaaggcgggagtggagaccaccacaccctccaaacaaagcaacaacaagtacgcggccagcagctatctgagcctgacgcctgagcagtggaagtcccacagaagctacagctgccaggtcacgcatgaagggagcaccgtggagaagacagtggcccctacagaatgttcataa

SEQ ID NO: 81 - DNA, 657 bp, Artificial Sequence
  Nucleic acid 2F4 VLCL2 CEA (AC25)
cagtctgtgttgacgcagccgccctcagtgtctgcggccccaggacagaaggtcaccatctcctgctctggaagcagctccaacattggtattacgcctgtatcctggtaccagcagctcccaggaacagcccccaaactcctcatttattctaataattttcgaccctcagggattcctgaccgattctctggctccaagtctggcacgtcagccaccctgggcatcaccggactccagactggggacgaggccgattattactgcggaacatgggataggactggtcatgagattaggcctgtgttcggcggagggaccaagctgaccgtcctaggtcagcccaaggctgccccctcggtcactctgttcccgccctcctctgaggagcttcaagccaacaaggccacactggtgtgtctcataagtgacttctacccgggagccgtgacagtggcttggaaagcagatagcagccccgtcaaggcgggagtggagaccaccacaccctccaaacaaagcaacaacaagtacgcggccagcagctatctgagcctgacgcctgagcagtggaagtcccacagaagctacagctgccaggtcacgcatgaagggagcaccgtggagaagacagtggcccctacagaatgttcataa

SEQ ID NO: 82 - DNA, 660 bp, Artificial Sequence
  Nucleic acid 2F7 VLCL2 CEA
cagtctgccctgactcagcctgcctccgtgtctgggtctcctggacagtcgatcaccatctcctgcactggaaccagcagtgacgttaagtatgcgaatgcggtctcctggtaccaacagcacccaggcaaagcccccaaactcatgatttattctaatagtattcggccctcaggggtttctaatcgcttctctggctccaagtctggcaacacggcctccctgaccatctctgggctccaggctgaggacgaggctgattattactgcagctcatatgatccccggggcaacctcctgatcagggtgttcggcggagggaccaagctgaccgtcctaggtcagcccaaggctgccccctcggtcactctgttcccgccctcctctgaggagcttcaagccaacaaggccacactggtgtgtctcataagtgacttctacccgggagccgtgacagtggcttggaaagcagatagcagccccgtcaaggcgggagtggagaccaccacaccctccaaacaaagcaacaacaagtacgcggccagcagctatctgagcctgacgcctgagcagtggaagtcccacagaagctacagctgccaggtcacgcatgaagggagcaccgtggagaagacagtggcccctacagaatgttcataa

SEQ ID NO: 83 - DNA, 657 bp, Artificial Sequence
  Nucleic acid 2C11 VLCL2 CEA (AC27)
cagtctgtgctgacgcagccgccctcagtgtctggggccccagggcagagggtcaccatctcctgcactgggagcagctccaacatcggttatgctgataaggtacactggtaccagcagcttccaggaacagcccccaaactcctcatctataataatagcgatcggccctcaggggtccctgaccgattctctggctccaagtctggcacctcagcctccctggccatcactgggctccaggctgaggatgaggctgattattactgccagtcctatgatggctacaacatgctgactgctgtgttcggcggagggaccaagctgaccgtcctaggtcagcccaaggctgccccctcggtcactctgttcccgccctcctctgaggagcttcaagccaacaaggccacactggtgtgtctcataagtgacttctacccgggagccgtgacagtggcttggaaagcagatagcagccccgtcaaggcgggagtggagaccaccacaccctccaaacaaagcaacaacaagtacgcggccagcagctatctgagcctgacgcctgagcagtggaagtcccacagaagctacagctgccaggtcacgcatgaagggagcaccgtggagaagacagtggcccctacagaatgttcataa

SEQ ID NO: 84 - DNA, 657 bp, Artificial Sequence
  Nucleic acid C11 VLCL2 CEA (AC28)
aattttatgctgactcagccccactctgtgtcggagtctccggggaagacggtaaccatctcctgcacccgcagcagtggcagcatcaatgatattacggtgcattggtaccagcagcgcccgggcagttcccccaccactgtgatctatgggtataacgcgagaccctctggggtccctgatcggttctctggctccatcgacagctcctccaactctgcctccctcaccatctctggactgaagactgaggacgaggctgactactactgtcagtcctgggatgggcatggttctgcgtatgtgttcggcggagggaccaagctgaccgtcctaggtcagcccaaggctgccccctcggtcactctgttcccgccctcctctgaggagcttcaagccaacaaggccacactggtgtgtctcataagtgacttctacccgggagccgtgacagtggcttggaaagcagatagcagccccgtcaaggcgggagtggagaccaccacaccctccaaacaaagcaacaacaagtacgcggccagcagctatctgagcctgacgcctgagcagtggaagtcccacagaagctacagctgccaggtcacgcatgaagggagcaccgtggagaagacagtggcccctacagaatgttcataa

SEQ ID NO: 85 - DNA, 660 bp, Artificial Sequence
  Nucleic acid 2B5 VLCL2 CEA (AC29)
cagtctgccctgactcagcctgcctccgtgtctgggtctcctggacagtcgatcaccatctcctgcactggaaccagcagtgacgttgagtttacgaatggtgtctcctggtaccaacagcacccaggcaaagcccccaaactcatgatttatggttttagtagtcggccctcaggggtttctaatcgcttctctggctccaagtctggcaacacggcctccctgaccatctctgggctccaggctgaggacgaggctgattattactgcagctcatatgatcccccctggcacctgctggctagggtgttcggcggagggaccaagctgaccgtcctaggtcagcccaaggctgccccctcggtcactctgttcccgccctcctctgaggagcttcaagccaacaaggccacactggtgtgtctcataagtgacttctacccgggagccgtgacagtggcttggaaagcagatagcagccccgtcaaggcgggagtggagaccaccacaccctccaaacaaagcaacaacaagtacgcggccagcagctatctgagcctgacgcctgagcagtggaagtcccacagaagctacagctgccaggtcacgcatgaagggagcaccgtggagaagacagtggcccctacagaatgttcataa

SEQ ID NO: 86 - DNA, 2109 bp, Homo sapiens
atggagtctccctcggcccctccccacagatggtgcatcccctggcagaggctcctgctcacagcctcacttctaaccttctggaacccgcccaccactgccaagctcactattgaatccacgccgttcaatgtcgcagaggggaaggaggtgcttctacttgtccacaatctgccccagcatctttttggctacagctggtacaaaggtgaaagagtggatggcaaccgtcaaattataggatatgtaataggaactcaacaagctaccccagggcccgcatacagtggtcgagagataatataccccaatgcatccctgctgatccagaacatcatccagaatgacacaggattctacaccctacacgtcataaagtcagatcttgtgaatgaagaagcaactggccagttccgggtatacccggagctgcccaagccctccatctccagcaacaactccaaacccgtggaggacaaggatgctgtggccttcacctgtgaacctgagactcaggacgcaacctacctgtggtgggtaaacaatcagagcctcccggtcagtcccaggctgcagctgtccaatggcaacaggaccctcactctattcaatgtcacaagaaatgacacagcaagctacaaatgtgaaacccagaacccagtgagtgccaggcgcagtgattcagtcatcctgaatgtcctctatggcccggatgcccccaccatttcccctctaaacacatcttacagatcaggggaaaatctgaacctctcctgccacgcagcctctaacccacctgcacagtactcttggtttgtcaatgggactttccagcaatccacccaagagctctttatccccaacatcactgtgaataatagtggatcctatacgtgccaagcccataactcagacactggcctcaataggaccacagtcacgacgatcacagtctatgcagagccacccaaacccttcatcaccagcaacaactccaaccccgtggaggatgaggatgctgtagccttaacctgtgaacctgagattcagaacacaacctacctgtggtgggtaaataatcagagcctcccggtcagtcccaggctgcagctgtccaatgacaacaggaccctcactctactcagtgtcacaaggaatgatgtaggaccctatgagtgtggaatccagaacaaattaagtgttgaccacagcgacccagtcatcctgaatgtcctctatggcccagacgaccccaccatttccccctcatacacctattaccgtccaggggtgaacctcagcctctcctgccatgcagcctctaacccacctgcacagtattcttggctgattgatgggaacatccagcaacacacacaagagctctttatctccaacatcactgagaagaacagcggactctatacctgccaggccaataactcagccagtggccacagcaggactacagtcaagacaatcacagtctctgcggagctgcccaagccctccatctccagcaacaactccaaacccgtggaggacaaggatgctgtggccttcacctgtgaacctgaggctcagaacacaacctacctgtggtgggtaaatggtcagagcctcccagtcagtcccaggctgcagctgtccaatggcaacaggaccctcactctattcaatgtcacaagaaatgacgcaagagcctatgtatgtggaatccagaactcagtgagtgcaaaccgcagtgacccagtcaccctggatgtcctctatgggccggacacccccatcatttcccccccagactcgtcttacctttcgggagcgaacctcaacctctcctgccactcggcctctaacccatccccgcagtattcttggcgtatcaatgggataccgcagcaacacacacaagttctctttatcgccaaaatcacgccaaataataacgggacctatgcctgttttgtctctaacttggctactggccgcaataattccatagtcaagagcatcacagtctctgcatctggaacttctcctggtctctcagctggggccactgtcggcatcatgattggagtgctggttggggttgctctgatataa

SEQ ID NO: 87 - protein, 702 aa, Homo sapiens
MESPSAPPHRWCIPWQRLLLTASLLTFWNPPTTAKLTIESTPFNVAEGKEVLLLVHNLPQHLFGYSWYKGERVDGNRQIIGYVIGTQQATPGPAYSGREIIYPNASLLIQNIIQNDTGFYTLHVIKSDLVNEEATGQFRVYPELPKPSISSNNSKPVEDKDAVAFTCEPETQDATYLWWVNNQSLPVSPRLQLSNGNRTLTLFNVTRNDTASYKCETQNPVSARRSDSVILNVLYGPDAPTISPLNTSYRSGENLNLSCHAASNPPAQYSWFVNGTFQQSTQELFIPNITVNNSGSYTCQAHNSDTGLNRTTVTTITVYAEPPKPFITSNNSNPVEDEDAVALTCEPEIQNTTYLWWVNNQSLPVSPRLQLSNDNRTLTLLSVTRNDVGPYECGIQNKLSVDHSDPVILNVLYGPDDPTISPSYTYYRPGVNLSLSCHAASNPPAQYSWLIDGNIQQHTQELFISNITEKNSGLYTCQANNSASGHSRTTVKTITVSAELPKPSISSNNSKPVEDKDAVAFTCEPEAQNTTYLWWVNGQSLPVSPRLQLSNGNRTLTLFNVTRNDARAYVCGIQNSVSANRSDPVTLDVLYGPDTPIISPPDSSYLSGANLNLSCHSASNPSPQYSWRINGIPQQHTQVLFIAKITPNNNGTYACFVSNLATGRNNSIVKSITVSASGTSPGLSAGATVGIMIGVLVGVALI

SEQ ID NO: 88 - protein, 121 aa, Artificial Sequence
  MAB CEA1 VH
QVQLVQSGAEVKKPGSSVKVSCKASGFNIKDTYMHWVRQAPGQGLEWMGRIDPANGNSKYVPKFQGRVTITADTSTSTAYMELSSLRSEDTAVYYCAPFGYYVSDYAMAYWGQGTLVTVSS

SEQ ID NO: 89 - protein, 111 aa, Artificial Sequence
  MAB CEA1 VL
EIVLTQSPATLSLSPGERATLSCRAGESVDIFGVGFLHWYQQKPGQAPRLLIYRASNRATGIPARFSGSGSGTDFTLTISSLEPEDFAVYYCQQTNEDPYTFGQGTKLEIK

SEQ ID NO: 90 - protein, 125 aa, Artificial Sequence
  MAB CD3 VH
EVQLLESGGGLVQPGGSLRLSCAASGFTFSTYAMNWVRQAPGKGLEWVSRIRSKYNNYATYYADSVKGRFTISRDDSKNTLYLQMNSLRAEDTAVYYCVRHGNFGNSYVSWFAYWGQGTLVTVSS

SEQ ID NO: 91 - protein, 109 aa, Artificial Sequence
  MAB CD3 VL
QAVVTQEPSLTVSPGGTVTLTCGSSTGAVTTSNYANWVQEKPGQAFRGLIGGTNKRAPGTPARFSGSLLGGKAALTLSGAQPEDEAEYYCALWYSNLWVFGGGTKLTVL

SEQ ID NO: 92 - protein, 232 aa, Artificial Sequence
  CD3 VH-CL(CK)
EVQLLESGGGLVQPGGSLRLSCAASGFTFSTYAMNWVRQAPGKGLEWVSRIRSKYNNYATYYADSVKGRFTISRDDSKNTLYLQMNSLRAEDTAVYYCVRHGNFGNSYVSWFAYWGQGTLVTVSSASVAAPSVFIFPPSDEQLKSGTASVVCLLNNFYPREAKVQWKVDNALQSGNSQESVTEQDSKDSTYSLSSTLTLSKADYEKHKVYACEVTHQGLSSPVTKSFNRGEC

SEQ ID NO: 93 - protein, 449 aa, Artificial Sequence
  CEA VH-CH1(EE)-Fc (hole, P329G LALA)
QVQLVQSGAEVKKPGSSVKVSCKASGFNIKDTYMHWVRQAPGQGLEWMGRIDPANGNSKYVPKFQGRVTITADTSTSTAYMELSSLRSEDTAVYYCAPFGYYVSDYAMAYWGQGTLVTVSSASTKGPSVFPLAPSSKSTSGGTAALGCLVEDYFPEPVTVSWNSGALTSGVHTFPAVLQSSGLYSLSSVVTVPSSSLGTQTYICNVNHKPSNTKVDEKVEPKSCDKTHTCPPCPAPEAAGGPSVFLFPPKPKDTLMISRTPEVTCVVVDVSHEDPEVKFNWYVDGVEVHNAKTKPREEQYNSTYRVVSVLTVLHQDWLNGKEYKCKVSNKALGAPIEKTISKAKGQPREPQVCTLPPSRDELTKNQVSLSCAVKGFYPSDIAVEWESNGQPENNYKTTPPVLDSDGSFFLVSKLTVDKSRWQQGNVFSCSVMHEALHNHYTQKSLSLSP

SEQ ID NO: 94 - protein, 614 aa, Artificial Sequence
  CEA VH-CH1(EE)-CD3 VL-CH1-Fc (knob, P329G LALA)
VPKFQGRVTITADTSTSTAYMELSSLRSEDTAVYYCAPFGYYVSDYAMAYWGQGTLVTVSSASTKGPSVFPLAPSSKSTSGGTAALGCLVEDYFPEPVTVSWNSGALTSGVHTFPAVLQSSGLYSLSSVVTVPSSSLGTQTYICNVNHKPSNTKVDEKVEPKSCDGGGGSGGGGSQAVVTQEPSLTVSPGGTVTLTCGSSTGAVTTSNYANWVQEKPGQAFRGLIGGTNKRAPGTPARFSGSLLGGKAALTLSGAQPEDEAEYYCALWYSNLWVFGGGTKLTVLSSASTKGPSVFPLAPSSKSTSGGTAALGCLVKDYFPEPVTVSWNSGALTSGVHTFPAVLQSSGLYSLSSVVTVPSSSLGTQTYICNVNHKPSNTKVDKKVEPKSCDKTHTCPPCPAPEAAGGPSVFLFPPKPKDTLMISRTPEVTCVVVDVSHEDPEVKFNWYVDGVEVHNAKTKPREEQYNSTYRVVSVLTVLHQDWLNGKEYKCKVSNKALGAPIEKTISKAKGQPREPQVYTLPPCRDELTKNQVSLWCLVKGFYPSDIAVEWESNGQPENNYKTTPPVLDSDGSFFLYSKLTVDKSRWQQGNVFSCSVMHEALHNHYTQKSLSLSP

SEQ ID NO: 95 - protein, 218 aa, Artificial Sequence
  CEA VL-CL(RK)
EIVLTQSPATLSLSPGERATLSCRAGESVDIFGVGFLHWYQQKPGQAPRLLIYRASNRATGIPARFSGSGSGTDFTLTISSLEPEDFAVYYCQQTNEDPYTFGQGTKLEIKRTVAAPSVFIFPPSDRKLKSGTASVVCLLNNFYPREAKVQWKVDNALQSGNSQESVTEQDSKDSTYSLSSTLTLSKADYEKHKVYACEVTHQGLSSPVTKSFNRGEC

SEQ ID NO: 96 - protein, 214 aa, Artificial Sequence
  LC CD3 CH2527 Cross Fab VL-CH1
QAVVTQEPSLTVSPGGTVTLTCGSSTGAVTTSNYANWVQEKPGQAFRGLIGGTNKRAPGTPARFSGSLLGGKAALTLSGAQPEDEAEYYCALWYSNLWVFGGGTKLTVLSSASTKGPSVFPLAPSSKSTSGGTAALGCLVKDYFPEPVTVSWNSGALTSGVHTFPAVLQSSGLYSLSSVVTVPSSSLGTQTYICNVNHKPSNTKVDKKVEPKSC

SEQ ID NO: 97 - protein, 451 aa, Artificial Sequence
  CEA CH1A10 VH CH1 FC Hole P329G LALA
QVQLVQSGAEVKKPGASVKVSCKASGYTFTEFGMNWVRQAPGQGLEWMGWINTKTGEATYVEEFKGRVTFTTDTSTSTAYMELRSLRSDDTAVYYCARWDFAYYVEAMDYWGQGTTVTVSSASTKGPSVFPLAPSSKSTSGGTAALGCLVKDYFPEPVTVSWNSGALTSGVHTFPAVLQSSGLYSLSSVVTVPSSSLGTQTYICNVNHKPSNTKVDKKVEPKSCDKTHTCPPCPAPEAAGGPSVFLFPPKPKDTLMISRTPEVTCVVVDVSHEDPEVKFNWYVDGVEVHNAKTKPREEQYNSTYRVVSVLTVLHQDWLNGKEYKCKVSNKALGAPIEKTISKAKGQPREPQVCTLPPSRDELTKNQVSLSCAVKGFYPSDIAVEWESNGQPENNYKTTPPVLDSDGSFFLVSKLTVDKSRWQQGNVFSCSVMHEALHNHYTQKSLSLSPGK

SEQ ID NO: 98 - protein, 694 aa, Artificial Sequence
  CEA CH1A1A CD3 CH2527 Cross Fab VH-CK FC Knob P329G LALA
QVQLVQSGAEVKKPGASVKVSCKASGYTFTEFGMNWVRQAPGQGLEWMGWINTKTGEATYVEEFKGRVTFTTDTSTSTAYMELRSLRSDDTAVYYCARWDFAYYVEAMDYWGQGTTVTVSSASTKGPSVFPLAPSSKSTSGGTAALGCLVKDYFPEPVTVSWNSGALTSGVHTFPAVLQSSGLYSLSSVVTVPSSSLGTQTYICNVNHKPSNTKVDKKVEPKSCDGGGGSGGGGSEVQLLESGGGLVQPGGSLRLSCAASGFTFSTYAMNWVRQAPGKGLEWVSRIRSKYNNYATYYADSVKGRFTISRDDSKNTLYLQMNSLRAEDTAVYYCVRHGNFGNSYVSWFAYWGQGTLVTVSSASVAAPSVFIFPPSDEQLKSGTASVVCLLNNFYPREAKVQWKVDNALQSGNSQESVTEQDSKDSTYSLSSTLTLSKADYEKHKVYACEVTHQGLSSPVTKSFNRGECDKTHTCPPCPAPEAAGGPSVFLFPPKPKDTLMISRTPEVTCVVVDVSHEDPEVKFNWYVDGVEVHNAKTKPREEQYNSTYRVVSVLTVLHQDWLNGKEYKCKVSNKALGAPIEKTISKAKGQPREPQVYTLPPCRDELTKNQVSLWCLVKGFYPSDIAVEWESNGQPENNYKTTPPVLDSDGSFFLYSKLTVDKSRWQQGNVFSCSVMHEALHNHYTQKSLSLSPGK

SEQ ID NO: 99 - protein, 215 aa, Artificial Sequence
  LC CEA 2F1 84
DIQMTQSPSSLSASVGDRVTITCKASAAVGTYVAWYQQKPGKAPKLLIYSASYRKRGVPSRFSGSGSGTDFTLTISSLQPEDFATYYCHQYYTYPLFTFGQGTKLEIKRTVAAPSVFIFPPSDEQLKSGTASVVCLLNNFYPREAKVQWKVDNALQSGNSQESVTEQDSKDSTYSLSSTLTLSKADYEKHKVYACEVTHQGLSSPVTKSFNRGEC

SEQ ID NO: 100 - protein, 106 aa, Artificial Sequence
  VK_SM3E
ENVLTQSPSSMSVSVGDRVNIACSASSSVPYMHWLQQKPGKSPKLLIYLTSNLASGVPSRFSGSGSGTDYSLTISSVQPEDAATYYCQQRSSYPLTFGGGTKLEIK

SEQ ID NO: 101 - protein, 120 aa, Artificial Sequence
  VH_SM3E
QVKLEQSGAEVVKPGASVKLSCKASGFNIKDSYMHWLRQGPGQRLEWIGWIDPENGDTEYAPKFQGKATFTTDTSANTAYLGLSSLRPEDTAVYYCNEGTPTGPYYFDYWGQGTLVTVSS

SEQ ID NO: 102 - protein, 116 aa, Artificial Sequence
  VL_MEDI
QAVLTQPASLSASPGASASLTCTLRRGINVGAYSIYWYQQKPGSPPQYLLRYKSDSDKQQGSGVSSRFSASKDASANAGILLISGLQSEDEADYYCMIWHSGASAVFGGGTKLTVL

SEQ ID NO: 103 - protein, 121 aa, Artificial Sequence
  VH_MEDI
EVQLVESGGGLVQPGRSLRLSCAASGFTVSSYWMHWVRQAPGKGLEWVGFIRNKANGGTTEYAASVKGRFTISRDDSKNTLYLQMNSLRAEDTAVYYCARDRGLRFYFDYWGQGTTVTVSS

SEQ ID NO: 104 - protein, 107 aa, Artificial Sequence
  VK_SAR
DIQMTQSPSSLSASVGDRVTITCRASENIFSYLAWYQQKPGKAPKLLIYNTRTLQSGVPSRFSGSGSGTDFTLTISSLQPEDFATYYCQHHYGTPFTFGQGTKLEIK

SEQ ID NO: 105 - protein, 120 aa, Artificial Sequence
  VH_SAR
EVQLVESGGGLVQPGGSLRLSCAASGFVFSSYDMSWVRQAPGKGLEWVSYISSGGGITYYADSVKGRFTISRDNSKNTLYLQMNSLRAEDTAVYYCAAHYFGSSGPFAYWGQGTLVTVSS

SEQ ID NO: 106 - protein, 108 aa, Artificial Sequence; identical to SEQ ID NO: 21
  VK_CH1A1A

SEQ ID NO: 107 - protein, 121 aa, Artificial Sequence; identical to SEQ ID NO: 20
  VH_ CH1A1A

SEQ ID NO: 108 - protein, 111 aa, Artificial Sequence; identical to SEQ ID NO: 89
  VK_T84.66

SEQ ID NO: 109 - protein, 121 aa, Artificial Sequence; identical to SEQ ID NO: 88
  VH_T84.66

SEQ ID NO: 110 - protein, 106 aa, Artificial Sequence
  VK_LABETUZUMAB
DIQLTQSPSSLSASVGDRVTITCKASQDVGTSVAWYQQKPGKAPKLLIYWTSTRHTGVPSRFSGSGSGTDFTFTISSLQPEDIATYYCQQYSLYRSFGQGTKVEIK

SEQ ID NO: 111 - protein, 119 aa, Artificial Sequence
  VH_LABETUZUMAB
EVQLVESGGGVVQPGRSLRLSCSASGFDFTTYWMSWVRQAPGKGLEWIGEIHPDSSTINYAPSLKDRFTISRDNAKNTLFLQMDSLRPEDTGVYFCASLYFGFPWFAYWGQGTPVTVSS

SEQ ID NO: 112 - protein, 13 aa, Artificial Sequence
  Mab CEA 1B2 (AC39) CDRL1
SGSSSEITASGVS

SEQ ID NO: 113 - protein, 7 aa, Artificial Sequence
  Mab CEA 1B2 (AC39) CDRL2
DNNKRPS

SEQ ID NO: 114 - protein, 11 aa, Artificial Sequence
  Mab CEA 1B2 (AC39) CDRL3
GTWDFPPSRFV

SEQ ID NO: 115 - protein, 216 aa, Artificial Sequence
  Mab CEA 1B2 (AC39) VLCL2
QSVLTQPPSVSAAPGQKVTISCSGSSSEITASGVSWYQQLPGTAPKLLIYDNNKRPSGIPDRFSGSKSGTSATLGITGLQTGDEADYYCGTWDFPPSRFVFGGGTKLTVLGQPKAAPSVTLFPPSSEELQANKATLVCLISDFYPGAVTVAWKADSSPVKAGVETTTPSKQSNNKYAASSYLSLTPEQWKSHRSYSCQVTHEGSTVEKTVAPTECS

SEQ ID NO: 116 - DNA, 651 bp, Artificial Sequence
  Mab CEA 1B2 (AC39) VLCL2, nucleic acid
cagtctgtgttgacgcagccgccctcagtgtctgcggccccaggacagaaggtcaccatctcctgctctggaagcagctccgagattactgcgtctggtgtatcctggtaccagcagctcccaggaacagcccccaaactcctcatttatgacaataataagcgaccctcagggattcctgaccgattctctggctccaagtctggcacgtcagccaccctgggcatcaccggactccagactggggacgaggccgattattactgcggaacatgggatttcccgccgtccaggttcgtgttcggcggagggaccaagctgaccgtcctaggtcagcccaaggctgccccctcggtcactctgttcccgccctcctctgaggagcttcaagccaacaaggccacactggtgtgtctcataagtgacttctacccgggagccgtgacagtggcttggaaagcagatagcagccccgtcaaggcgggagtggagaccaccacaccctccaaacaaagcaacaacaagtacgcggccagcagctatctgagcctgacgcctgagcagtggaagtcccacagaagctacagctgccaggtcacgcatgaagggagcaccgtggagaagacagtggcccctacagaatgttcataa